European Patent Application EP 4 357 781 A1, published April 24, 2024. Title: Immunoassay method and immunoassay kit for SARS-CoV-2. Applicant: Sekisui Medical Co., Ltd. The sequence listing filed with the application follows.

SEQUENCE LISTING (82 sequences)

SEQ ID NO: 1 - protein, 27 aa, Unknown
  SARS-CoV-2
KQQTVTLLPAADLDDFSKQLQQSMSSA

SEQ ID NO: 2 - protein, 18 aa, Unknown
  SARS-CoV-2
KQQTVTLLPAADLDDFSK

SEQ ID NO: 3 - protein, 18 aa, Unknown
  SARS-CoV-2
AADLDDFSKQLQQSMSSA

SEQ ID NO: 4 - protein, 10 aa, Unknown
  S32213HCCDR1
GFSLSTSGMG

SEQ ID NO: 5 - protein, 7 aa, Unknown
  S32213HCCDR2
IYWDDDK

SEQ ID NO: 6 - protein, 11 aa, Unknown
  S32213HCCDR3
ARRDYGYNFDY

SEQ ID NO: 7 - protein, 7 aa, Unknown
  S32213LCCDR1
SSVSSTY

SEQ ID NO: 8 - protein, 3 aa, Unknown
  S32213LCCDR2
STS

SEQ ID NO: 9 - protein, 9 aa, Unknown
  S32213LCCDR3
HQWSSYPPT

SEQ ID NO: 10 - protein, 8 aa, Unknown
  S32217HCCDR1
GFTFSDYY

SEQ ID NO: 11 - protein, 8 aa, Unknown
  S32217HCCDR2
ITDGDNYT

SEQ ID NO: 12 - protein, 14 aa, Unknown
  S32217HCCDR3
ARDGNYYASSPFTY

SEQ ID NO: 13 - protein, 9 aa, Unknown
  S32217LCCDR1
TGAVTTSNY

SEQ ID NO: 14 - protein, 3 aa, Unknown
  S32217LCCDR2
GTN

SEQ ID NO: 15 - protein, 9 aa, Unknown
  S32217LCCDR3
ALWYSNHWV

SEQ ID NO: 16 - protein, 8 aa, Unknown
  S32223HCCDR1
GFTFSDYY

SEQ ID NO: 17 - protein, 8 aa, Unknown
  S32223HCCDR2
ISDGYSYT

SEQ ID NO: 18 - protein, 13 aa, Unknown
  S32223HCCDR3
ARDQDYFGSSLAY

SEQ ID NO: 19 - protein, 9 aa, Unknown
  S32223LCCDR1
TGAVTTSNY

SEQ ID NO: 20 - protein, 3 aa, Unknown
  S32223LCCDR2
GTN

SEQ ID NO: 21 - protein, 9 aa, Unknown
  S32223LCCDR3
ALWYSNRWV

SEQ ID NO: 22 - protein, 419 aa, Unknown
  SARS-CoV-2
MSDNGPQNQRNAPRITFGGPSDSTGSNQNGERSGARSKQRRPQGLPNNTASWFTALTQHGKEDLKFPRGQGVPINTNSSPDDQIGYYRRATRRIRGGDGKMKDLSPRWYFYYLGTGPEAGLPYGANKDGIIWVATEGALNTPKDHIGTRNPANNAAIVLQLPQGTTLPKGFYAEGSRGGSQASSRSSSRSRNSSRNSTPGSSRGTSPARMAGNGGDAALALLLLDRLNQLESKMSGKGQQQQGQTVTKKSAAEASKKPRQKRTATKAYNVTQAFGRRGPEQTQGNFGDQELIRQGTDYKHWPQIAQFAPSASAFFGMSRIGMEVTPSGTWLTYTGAIKLDDKDPNFKDQVILLNKHIDAYKTFPPTEPKKDKKKKADETQALPQRQKKQQTVTLLPAADLDDFSKQLQQSMSSADSTQA

SEQ ID NO: 23 - protein, 174 aa, Unknown
  SARS-CoV-2
MSDNGPQNQRNAPRITFGGPSDSTGSNQNGERSGARSKQRRPQGLPNNTASWFTALTQHGKEDLKFPRGQGVPINTNSSPDDQIGYYRRATRRIRGGDGKMKDLSPRWYFYYLGTGPEAGLPYGANKDGIIWVATEGALNTPKDHIGTRNPANNAAIVLQLPQGTTLPKGFYAE

SEQ ID NO: 24 - protein, 73 aa, Unknown
  SARS-CoV-2
GSRGGSQASSRSSSRSRNSSRNSTPGSSRGTSPARMAGNGGDAALALLLLDRLNQLESKMSGKGQQQQGQTVT

SEQ ID NO: 25 - protein, 172 aa, Unknown
  SARS-CoV-2
KKSAAEASKKPRQKRTATKAYNVTQAFGRRGPEQTQGNFGDQELIRQGTDYKHWPQIAQFAPSASAFFGMSRIGMEVTPSGTWLTYTGAIKLDDKDPNFKDQVILLNKHIDAYKTFPPTEPKKDKKKKADETQALPQRQKKQQTVTLLPAADLDDFSKQLQQSMSSADSTQA

SEQ ID NO: 26 - protein, 5 aa, Unknown
  SARS-CoV-2
LLPAA

SEQ ID NO: 27 - protein, 9 aa, Unknown
  SARS-CoV-2
LDDFSKQLQ

SEQ ID NO: 28 - protein, 18 aa, Unknown
  peptide 1
ARMAGNGGDAALALLLLD

SEQ ID NO: 29 - protein, 19 aa, Unknown
  peptide 2
TAALALLLLDRLNQLESKM

SEQ ID NO: 30 - protein, 18 aa, Unknown
  peptide 3
RLNQLESKMSGKGQQQQG

SEQ ID NO: 31 - protein, 18 aa, Unknown
  peptide 4
SGKGQQQQGQTVTKKSAA

SEQ ID NO: 32 - protein, 18 aa, Unknown
  peptide 5
QTVTKKSAAEASKKPRQK

SEQ ID NO: 33 - protein, 18 aa, Unknown
  peptide 6
EASKKPRQKRTATKAYNV

SEQ ID NO: 34 - protein, 18 aa, Unknown
  peptide 7
RTATKAYNVTQAFGRRGP

SEQ ID NO: 35 - protein, 18 aa, Unknown
  peptide 8
TQAFGRRGPEQTQGNFGD

SEQ ID NO: 36 - protein, 18 aa, Unknown
  peptide 9
EQTQGNFGDQELIRQGTD

SEQ ID NO: 37 - protein, 18 aa, Unknown
  peptide 10
QELIRQGTDYKHWPQIAQ

SEQ ID NO: 38 - protein, 18 aa, Unknown
  peptide 11
YKHWPQIAQFAPSASAFF

SEQ ID NO: 39 - protein, 18 aa, Unknown
  peptide 12
FAPSASAFFGMSRIGMEV

SEQ ID NO: 40 - protein, 18 aa, Unknown
  peptide 13
GMSRIGMEVTPSGTWLTY

SEQ ID NO: 41 - protein, 18 aa, Unknown
  peptide 14
TPSGTWLTYTGAIKLDDK

SEQ ID NO: 42 - protein, 18 aa, Unknown
  peptide 15
TGAIKLDDKDPNFKDQVI

SEQ ID NO: 43 - protein, 18 aa, Unknown
  peptide 16
DPNFKDQVILLNKHIDAY

SEQ ID NO: 44 - protein, 19 aa, Unknown
  peptide 17
LLNKHIDAYKITFPPTEPK

SEQ ID NO: 45 - protein, 18 aa, Unknown
  peptide 18
KTFPPTEPKKDKKKKADE

SEQ ID NO: 46 - protein, 18 aa, Unknown
  peptide 19
KDKKKKADETQALPQRQK

SEQ ID NO: 47 - protein, 18 aa, Unknown
  peptide 20
TQALPQRQKKQQTVTLLP

SEQ ID NO: 48 - protein, 18 aa, Unknown
  peptide 21
KQQTVTLLPAADLDDFSK

SEQ ID NO: 49 - protein, 18 aa, Unknown
  peptide 22
AADLDDFSKQLQQSMSSA

SEQ ID NO: 50 - protein, 14 aa, Unknown
  peptide 23
QLQQSMSSADSTQA

SEQ ID NO: 51 - protein, 7 aa, Unknown
  peptide 24
RQKKQQT

SEQ ID NO: 52 - protein, 7 aa, Unknown
  peptide 25
QKKQQTV

SEQ ID NO: 53 - protein, 7 aa, Unknown
  peptide 26
KKQQTVT

SEQ ID NO: 54 - protein, 7 aa, Unknown
  peptide 27
KQQTVTL

SEQ ID NO: 55 - protein, 7 aa, Unknown
  peptide 28
QQTVTLL

SEQ ID NO: 56 - protein, 7 aa, Unknown
  peptide 29
QTVTLLP

SEQ ID NO: 57 - protein, 7 aa, Unknown
  peptide 30
TVTLLPA

SEQ ID NO: 58 - protein, 7 aa, Unknown
  peptide 31
VTLLPAA

SEQ ID NO: 59 - protein, 7 aa, Unknown
  peptide 32
TLLPAAD

SEQ ID NO: 60 - protein, 7 aa, Unknown
  peptide 33
LLPAADL

SEQ ID NO: 61 - protein, 7 aa, Unknown
  peptide 34
LPAADLD

SEQ ID NO: 62 - protein, 7 aa, Unknown
  peptide 35
PAADLDD

SEQ ID NO: 63 - protein, 7 aa, Unknown
  peptide 36
AADIDDF

SEQ ID NO: 64 - protein, 7 aa, Unknown
  peptide 37
ADLDDFS

SEQ ID NO: 65 - protein, 7 aa, Unknown
  peptide 38
DLDDESK

SEQ ID NO: 66 - protein, 7 aa, Unknown
  peptide 39
LDDFSKQ

SEQ ID NO: 67 - protein, 15 aa, Unknown
  peptide 40
QQTVTLLPAADLDDF

SEQ ID NO: 68 - protein, 15 aa, Unknown
  ptide 41
QTVTLLPAADLDDFS

SEQ ID NO: 69 - protein, 15 aa, Unknown
  eptide 42
TVTLLPAADLDDFSK

SEQ ID NO: 70 - protein, 15 aa, Unknown
  peptide 43
VTLLPAADLDDESKQ

SEQ ID NO: 71 - protein, 15 aa, Unknown
  peptide 44
TLLPAADLDDFSKQL

SEQ ID NO: 72 - protein, 15 aa, Unknown
  peptide 45
LLPAADLDDESKQLQ

SEQ ID NO: 73 - protein, 15 aa, Unknown
  peptide 46
LPAADLDDFSKQLQQ

SEQ ID NO: 74 - protein, 15 aa, Unknown
  peptide 47
PAADLDDFSKQLQQS

SEQ ID NO: 75 - protein, 15 aa, Unknown
  peptide 48
PAADLDDFSKQLQQS

SEQ ID NO: 76 - protein, 15 aa, Unknown
  peptide 49
ADLDDFSKQLQQSMS

SEQ ID NO: 77 - protein, 15 aa, Unknown
  peptide 50
DLDDFSKQLQQSMSS

SEQ ID NO: 78 - protein, 15 aa, Unknown
  peptide 51
LDDFSKQLQQSMSSA

SEQ ID NO: 79 - protein, 15 aa, Unknown
  peptide 52
DDFSKQLQQSMSSAD

SEQ ID NO: 80 - protein, 15 aa, Unknown
  peptide 53
DFSKQLQQSMSSADS

SEQ ID NO: 81 - protein, 15 aa, Unknown
  peptide 54
FSKQLQQSMSSADST

SEQ ID NO: 82 - protein, 15 aa, Unknown
  peptide 55
SKQLQQSMSSADSTQ